European Patent Application EP 4 715 041 A1, published March 25, 2026. Title: HIGH-THROUGHPUT FABRICATION OF STRATIFIED CO-CULTURES. Applicant: L V M H RECHERCHE. The sequence listing filed with the application follows.

SEQUENCE LISTING (12 sequences)

SEQ ID NO: 1 - DNA, 20 bp, synthetic construct
  source 1..20: mol_type = other DNA; note = Forward primer for keratin 1
tgacaaggtgaggttcctgg

SEQ ID NO: 2 - DNA, 20 bp, synthetic construct
  source 1..20: mol_type = other DNA; note = Reverse primer for keratin 1
gttggtccactctccttcgg

SEQ ID NO: 3 - DNA, 24 bp, synthetic construct
  source 1..24: mol_type = other DNA; note = Forward primer for keratin 10
tgatgtgaatgtggaaatgaatgc

SEQ ID NO: 4 - DNA, 24 bp, synthetic construct
  source 1..24: mol_type = other DNA; note = Reverse primer for keratin 10
gtagtcagttccttgctcttttca

SEQ ID NO: 5 - DNA, 20 bp, synthetic construct
  source 1..20: mol_type = other DNA; note = Forward primer for collagen VII A1
aaggacctcggggagacaat

SEQ ID NO: 6 - DNA, 20 bp, synthetic construct
  source 1..20: mol_type = other DNA; note = Reverse primer for collagen VII A1
cggataccaggcactccatc

SEQ ID NO: 7 - DNA, 20 bp, synthetic construct
  source 1..20: mol_type = other DNA; note = Forward primer of involucrin
ctgcctcagccttactgtga

SEQ ID NO: 8 - DNA, 21 bp, synthetic construct
  source 1..21: mol_type = other DNA; note = Reverse primer for involucrin
ggaggaggaacagtcttgagg

SEQ ID NO: 9 - DNA, 20 bp, synthetic construct
  source 1..20: mol_type = other DNA; note = Forward primer for loricrin
gcaaacctcgggtagcatca

SEQ ID NO: 10 - DNA, 20 bp, synthetic construct
  source 1..20: mol_type = other DNA; note = Reverse primer for loricrin
gccgtccaaatagatccccc

SEQ ID NO: 11 - DNA, 21 bp, synthetic construct
  source 1..21: mol_type = other DNA; note = Forward primer for GAPDH
atcaagaaggtggtgaagcag

SEQ ID NO: 12 - DNA, 20 bp, synthetic construct
  source 1..20: mol_type = other DNA; note = Reverse primer for GAPDH
gtcgctgttgaagtcagagg